European Patent Application EP 4 471 147 A1, published December 4, 2024. Title: Anti-SARS-CoV-2 Human Neutralizing Antibody With Mutant Crossover And Its Antigen-Binding Fragment. Applicant: Evec Incorporated. Application JP. The sequence listing filed with the application follows.

SEQUENCE LISTING (21 sequences)

SEQ ID NO: 1 - protein, 119 aa, Homo sapiens
EVQLVESGGGLIQPGGSLRLSCAASGLTVSSNYMSWVRQAPGKGLEWVSLIYPGGSTYYADSVKGRFTISRDNSNNTLYLRMNSLRAEDTAVYYCARDLPHIAATGRVSGQGTLVTVSS

SEQ ID NO: 2 - protein, 8 aa, Homo sapiens
GLTVSSNY

SEQ ID NO: 3 - protein, 7 aa, Homo sapiens
IYPGGST

SEQ ID NO: 4 - protein, 13 aa, Homo sapiens
ARDLPHIAATGRV

SEQ ID NO: 5 - protein, 107 aa, Homo sapiens
DIQMTQSPSSLSASVGDRVAITCQASQDINKYLNWYQQKPGKAPKLLIYDASNLETGVPSRFSGSGSGTDFTFTISSLQPEDFATYYCHQYDNLPPTFGPGTKVDIK

SEQ ID NO: 6 - protein, 6 aa, Homo sapiens
QDINKY

SEQ ID NO: 7 - skipped

SEQ ID NO: 8 - protein, 9 aa, Homo sapiens
HQYDNLPPT

SEQ ID NO: 9 - protein, 449 aa, Homo sapiens
EVQLVESGGGLIQPGGSLRLSCAASGLTVSSNYMSWVRQAPGKGLEWVSLIYPGGSTYYADSVKGRFTISRDNSNNTLYLRMNSLRAEDTAVYYCARDLPHIAATGRVSGQGTLVTVSSASTKGPSVFPLAPSSKSTSGGTAALGCLVKDYFPEPVTVSWNSGALTSGVHTFPAVLQSSGLYSLSSVVTVPSSSLGTQTYICNVNHKPSNTKVDKKVEPKSCDKTHTCPPCPAPELLGGPSVFLFPPKPKDTLMISRTPEVTCVVVDVSHEDPEVKFNWYVDGVEVHNAKTKPREEQYNSTYRVVSVLTVLHQDWLNGKEYKCKVSNKALPAPIEKTISKAKGQPREPQVYTLPPSRDELTKNQVSLTCLVKGFYPSDIAVEWESNGQPENNYKTTPPVLDSDGSFFLYSKLTVDKSRWQQGNVFSCSVMHEALHNHYTQKSLSLSPGK

SEQ ID NO: 10 - protein, 214 aa, Homo sapiens
DIQMTQSPSSLSASVGDRVAITCQASQDINKYLNWYQQKPGKAPKLLIYDASNLETGVPSRFSGSGSGTDFTFTISSLQPEDFATYYCHQYDNLPPTFGPGTKVDIKRTVAAPSVFIFPPSDEQLKSGTASVVCLLNNFYPREAKVQWKVDNALQSGNSQESVTEQDSKDSTYSLSSTLTLSKADYEKHKVYACEVTHQGLSSPVTKSFNRGEC

SEQ ID NO: 11 - protein, 119 aa, Homo sapiens
EVQLVESGGGLIQPGGSLRLSCAASGLTVSSNYMSWVRQAPGKGLEWVSLIYPGGSTYYADSVKGRFTISRDNSNNTLYLRMNSLRAEDTAVYYCARDLPHIAATGRVWGQGTLVTVSS

SEQ ID NO: 12 - protein, 449 aa, Homo sapiens
EVQLVESGGGLIQPGGSLRLSCAASGLTVSSNYMSWVRQAPGKGLEWVSLIYPGGSTYYADSVKGRFTISRDNSNNTLYLRMNSLRAEDTAVYYCARDLPHIAATGRVWGQGTLVTVSSASTKGPSVFPLAPSSKSTSGGTAALGCLVKDYFPEPVTVSWNSGALTSGVHTFPAVLQSSGLYSLSSVVTVPSSSLGTQTYICNVNHKPSNTKVDKKVEPKSCDKTHTCPPCPAPELLGGPSVFLFPPKPKDTLMISRTPEVTCVVVDVSHEDPEVKFNWYVDGVEVHNAKTKPREEQYNSTYRVVSVLTVLHQDWLNGKEYKCKVSNKALPAPIEKTISKAKGQPREPQVYTLPPSRDELTKNQVSLTCLVKGFYPSDIAVEWESNGQPENNYKTTPPVLDSDGSFFLYSKLTVDKSRWQQGNVFSCSVMHEALHNHYTQKSLSLSPGK

SEQ ID NO: 13 - DNA, 1350 bp, Homo sapiens
  source 1..1350: mol_type = genomic DNA
gaggtgcagctggtggagtctggaggaggcctgatccagcctggggggtccctgagactctcctgtgcagcctctggcttaaccgtcagtagcaactacatgagctgggtccgccaggctccagggaaggggctggagtgggtctcacttatttatcccggtggtagcacatactacgcagactccgtgaagggccgattcaccatctccagagacaattccaacaacacgctgtatcttcgaatgaacagcctgagagccgaggacacggccgtgtattactgtgcgagagatcttccccatatagccgcaactgggcgcgtctcgggccagggaaccctggtcaccgtctcctcagcctccaccaagggcccatcggtcttccccctggcaccctcctccaagagcacctctgggggcacagcggccctgggctgcctggtcaaggactacttccccgaaccggtgacggtgtcgtggaactcaggcgccctgaccagcggcgtgcacaccttcccggctgtcctacagtcctcaggactctactccctcagcagcgtggtgaccgtgccctccagcagcttgggcacccagacctacatctgcaacgtgaatcacaagcccagcaacaccaaggtggacaagaaagttgagcccaaatcttgtgacaaaactcacacatgcccaccgtgcccagcacctgaactcctggggggaccgtcagtcttcctcttccccccaaaacccaaggacaccctcatgatctcccggacccctgaggtcacatgcgtggtggtggacgtgagccacgaagaccctgaggtcaagttcaactggtacgtggacggcgtggaggtgcataatgccaagacaaagccgcgggaggagcagtacaacagcacgtaccgtgtggtcagcgtcctcaccgtcctgcaccaggactggctgaatggcaaggagtacaagtgcaaggtctccaacaaagccctcccagcccccatcgagaaaaccatctccaaagccaaagggcagccccgagaaccacaggtgtacaccctgcccccatcccgggatgagctgaccaagaaccaggtcagcctgacctgcctggtcaaaggcttctatcccagcgacatcgccgtggagtgggagagcaatgggcagccggagaacaactacaagaccacgcctcccgtgctggactccgacggctccttcttcctctacagcaagctcaccgtggacaagagcaggtggcagcaggggaacgtcttctcatgctccgtgatgcatgaggctctgcacaaccactacacgcagaagagcctctccctgtctccgggtaaatga

SEQ ID NO: 14 - DNA, 1350 bp, Homo sapiens
  source 1..1350: mol_type = genomic DNA
gaggtgcagctggtggagtctggaggaggcctgatccagcctggggggtccctgagactctcctgtgcagcctctggcttaaccgtcagtagcaactacatgagctgggtccgccaggctccagggaaggggctggagtgggtctcacttatttatcccggtggtagcacatactacgcagactccgtgaagggccgattcaccatctccagagacaattccaacaacacgctgtatcttcgaatgaacagcctgagagccgaggacacggccgtgtattactgtgcgagagatcttccccatatagccgcaactgggcgcgtctggggccagggaaccctggtcaccgtctcctcagcctccaccaagggcccatcggtcttccccctggcaccctcctccaagagcacctctgggggcacagcggccctgggctgcctggtcaaggactacttccccgaaccggtgacggtgtcgtggaactcaggcgccctgaccagcggcgtgcacaccttcccggctgtcctacagtcctcaggactctactccctcagcagcgtggtgaccgtgccctccagcagcttgggcacccagacctacatctgcaacgtgaatcacaagcccagcaacaccaaggtggacaagaaagttgagcccaaatcttgtgacaaaactcacacatgcccaccgtgcccagcacctgaactcctggggggaccgtcagtcttcctcttccccccaaaacccaaggacaccctcatgatctcccggacccctgaggtcacatgcgtggtggtggacgtgagccacgaagaccctgaggtcaagttcaactggtacgtggacggcgtggaggtgcataatgccaagacaaagccgcgggaggagcagtacaacagcacgtaccgtgtggtcagcgtcctcaccgtcctgcaccaggactggctgaatggcaaggagtacaagtgcaaggtctccaacaaagccctcccagcccccatcgagaaaaccatctccaaagccaaagggcagccccgagaaccacaggtgtacaccctgcccccatcccgggatgagctgaccaagaaccaggtcagcctgacctgcctggtcaaaggcttctatcccagcgacatcgccgtggagtgggagagcaatgggcagccggagaacaactacaagaccacgcctcccgtgctggactccgacggctccttcttcctctacagcaagctcaccgtggacaagagcaggtggcagcaggggaacgtcttctcatgctccgtgatgcatgaggctctgcacaaccactacacgcagaagagcctctccctgtctccgggtaaatga

SEQ ID NO: 15 - DNA, 645 bp, Homo sapiens
  source 1..645: mol_type = genomic DNA
gacatccagatgacccagtctccatcctccctgtctgcatctgtaggagacagagtcgccatcacttgccaggcgagtcaggacattaacaagtatttaaattggtatcagcagaaaccagggaaagcccctaagctcctgatctacgatgcatccaatttggaaacaggggtcccatcaaggttcagtggaagtggatctgggacagattttactttcaccatcagcagcctgcagcctgaagattttgcaacatattactgtcaccagtatgataatctccctccgactttcggccctgggaccaaagtggatatcaaacgaactgtggctgcaccatctgtcttcatcttcccgccatctgatgagcagttgaaatctggaactgcctctgttgtgtgcctgctgaataacttctatcccagagaggccaaagtacagtggaaggtggataacgccctccaatcgggtaactcccaggagagtgtcacagagcaggacagcaaggacagcacctacagcctcagcagcaccctgacgctgagcaaagcagactacgagaaacacaaagtctacgcctgcgaagtcacccatcagggcctgagctcgcccgtcacaaagagcttcaacaggggagagtgttag

SEQ ID NO: 16 - DNA, 1353 bp, Homo sapiens
  source 1..1353: mol_type = genomic DNA
gacgaggtgcagctggtggagtctggaggaggcctgatccagcctggggggtccctgagactctcctgtgcagcctctggcttaaccgtcagtagcaactacatgagctgggtccgccaggctccagggaaggggctggagtgggtctcacttatttatcccggtggtagcacatactacgcagactccgtgaagggccgattcaccatctccagagacaattccaacaacacgctgtatcttcgaatgaacagcctgagagccgaggacacggccgtgtattactgtgcgagagatcttccccatatagccgcaactgggcgcgtctggggccagggaaccctggtcaccgtctcctcagcctccaccaagggcccatcggtcttccccctggcaccctcctccaagagcacctctgggggcacagcggccctgggctgcctggtcaaggactacttccccgaaccggtgacggtgtcgtggaactcaggcgccctgaccagcggcgtgcacaccttcccggctgtcctacagtcctcaggactctactccctcagcagcgtggtgaccgtgccctccagcagcttgggcacccagacctacatctgcaacgtgaatcacaagcccagcaacaccaaggtggacaagaaagttgagcccaaatcttgtgacaaaactcacacatgcccaccgtgcccagcacctgaactcctggggggaccgtcagtcttcctcttccccccaaaacccaaggacaccctcatgatctcccggacccctgaggtcacatgcgtggtggtggacgtgagccacgaagaccctgaggtcaagttcaactggtacgtggacggcgtggaggtgcataatgccaagacaaagccgcgggaggagcagtacaacagcacgtaccgtgtggtcagcgtcctcaccgtcctgcaccaggactggctgaatggcaaggagtacaagtgcaaggtctccaacaaagccctcccagcccccatcgagaaaaccatctccaaagccaaagggcagccccgagaaccacaggtgtacaccctgcccccatcccgggatgagctgaccaagaaccaggtcagcctgacctgcctggtcaaaggcttctatcccagcgacatcgccgtggagtgggagagcaatgggcagccggagaacaactacaagaccacgcctcccgtgctggactccgacggctccttcttcctctacagcaagctcaccgtggacaagagcaggtggcagcaggggaacgtcttctcatgctccgtgatgcatgaggctctgcacaaccactacacgcagaagagcctctccctgtctccgggtaaatga

SEQ ID NO: 17 - protein, 450 aa, Homo sapiens
DEVQLVESGGGLIQPGGSLRLSCAASGLTVSSNYMSWVRQAPGKGLEWVSLIYPGGSTYYADSVKGRFTISRDNSNNTLYLRMNSLRAEDTAVYYCARDLPHIAATGRVWGQGTLVTVSSASTKGPSVFPLAPSSKSTSGGTAALGCLVKDYFPEPVTVSWNSGALTSGVHTFPAVLQSSGLYSLSSVVTVPSSSLGTQTYICNVNHKPSNTKVDKKVEPKSCDKTHTCPPCPAPELLGGPSVFLFPPKPKDTLMISRTPEVTCVVVDVSHEDPEVKFNWYVDGVEVHNAKTKPREEQYNSTYRVVSVLTVLHQDWLNGKEYKCKVSNKALPAPIEKTISKAKGQPREPQVYTLPPSRDELTKNQVSLTCLVKGFYPSDIAVEWESNGQPENNYKTTPPVLDSDGSFFLYSKLTVDKSRWQQGNVFSCSVMHEALHNHYTQKSLSLSPGK

SEQ ID NO: 18 - DNA, 648 bp, Homo sapiens
  source 1..648: mol_type = genomic DNA
gacgacatccagatgacccagtctccatcctccctgtctgcatctgtaggagacagagtcgccatcacttgccaggcgagtcaggacattaacaagtatttaaattggtatcagcagaaaccagggaaagcccctaagctcctgatctacgatgcatccaatttggaaacaggggtcccatcaaggttcagtggaagtggatctgggacagattttactttcaccatcagcagcctgcagcctgaagattttgcaacatattactgtcaccagtatgataatctccctccgactttcggccctgggaccaaagtggatatcaaacgaactgtggctgcaccatctgtcttcatcttcccgccatctgatgagcagttgaaatctggaactgcctctgttgtgtgcctgctgaataacttctatcccagagaggccaaagtacagtggaaggtggataacgccctccaatcgggtaactcccaggagagtgtcacagagcaggacagcaaggacagcacctacagcctcagcagcaccctgacgctgagcaaagcagactacgagaaacacaaagtctacgcctgcgaagtcacccatcagggcctgagctcgcccgtcacaaagagcttcaacaggggagagtgttag

SEQ ID NO: 19 - protein, 215 aa, Homo sapiens
DDIQMTQSPSSLSASVGDRVAITCQASQDINKYLNWYQQKPGKAPKLLIYDASNLETGVPSRFSGSGSGTDFTFTISSLQPEDFATYYCHQYDNLPPTFGPGTKVDIKRTVAAPSVFIFPPSDEQLKSGTASVVCLLNNFYPREAKVQWKVDNALQSGNSQESVTEQDSKDSTYSLSSTLTLSKADYEKHKVYACEVTHQGLSSPVTKSFNRGEC

SEQ ID NO: 20 - protein, 120 aa, Homo sapiens
DEVQLVESGGGLIQPGGSLRLSCAASGLTVSSNYMSWVRQAPGKGLEWVSLIYPGGSTYYADSVKGRFTISRDNSNNTLYLRMNSLRAEDTAVYYCARDLPHIAATGRVWGQGTLVTVSS

SEQ ID NO: 21 - protein, 108 aa, Homo sapiens
DDIQMTQSPSSLSASVGDRVAITCQASQDINKYLNWYQQKPGKAPKLLIYDASNLETGVPSRFSGSGSGTDFTFTISSLQPEDFATYYCHQYDNLPPTFGPGTKVDIK